European Patent Application EP 4 682 270 A1, published January 21, 2026. Title: Method for relative quantification of GM crop using digital PCR without CRM. Applicant: NEX BIO. Application KR. The sequence listing filed with the application follows.

SEQUENCE LISTING (12 sequences)

SEQ ID NO: 1 - DNA, 18 bp, synthetic construct
  source 1..18: mol_type = other DNA
tgggtgggcacattattt

SEQ ID NO: 2 - DNA, 18 bp, synthetic construct
  source 1..18: mol_type = other DNA
aacaacccctaacatcct

SEQ ID NO: 3 - DNA, 20 bp, synthetic construct
  source 1..20: mol_type = other DNA
acagctgacacaccatgtac

SEQ ID NO: 4 - DNA, 20 bp, synthetic construct
  source 1..20: mol_type = other DNA
aaaagaccacaacaagccgc

SEQ ID NO: 5 - DNA, 23 bp, synthetic construct
  source 1..23: mol_type = other DNA
caatgcgttctccaccaagtact

SEQ ID NO: 6 - DNA, 27 bp, synthetic construct
  source 1..27: mol_type = other DNA
cgaccatggacaacaacccaaacatca

SEQ ID NO: 7 - DNA, 21 bp, synthetic construct
  source 1..21: mol_type = other DNA
tggagtgaagtaatgcattgc

SEQ ID NO: 8 - DNA, 20 bp, synthetic construct
  source 1..20: mol_type = other DNA
attttactcccactgctgcc

SEQ ID NO: 9 - DNA, 27 bp, synthetic construct
  source 1..27: mol_type = other DNA
ttgtactaccgtgccattttgctaagt

SEQ ID NO: 10 - DNA, 24 bp, synthetic construct
  source 1..24: mol_type = other DNA
cctttaggatttcagcatcagtgg

SEQ ID NO: 11 - DNA, 18 bp, synthetic construct
  source 1..18: mol_type = other DNA
gacttgtcgccgggaatg

SEQ ID NO: 12 - DNA, 19 bp, synthetic construct
  source 1..19: mol_type = other DNA
cgcaaccgcccgcaaatcc